European Patent Specification EP 3 624 856 B1, published April 3, 2024. Title: GENE THERAPY FOR TUBEROUS SCLEROSIS. Applicant: The General Hospital Corporation. The sequence listing filed with the application follows.

SEQUENCE LISTING (12 sequences)

SEQ ID NO: 1 - protein, 758 aa, Artificial Sequence
  Synthetic Construct
MAKPTSKDSGLKEKFKILLGLGTPRPNPRSAEGKQTEFIITAEILRELSMECGLNNRIRMIGQICEVAKTKKFEEHAVEALWKAVADLLQPERPLEARHAVLALLKAIVQGQGERLGVLRALFFKVIKDYPSNEDLHERLEVFKALTDNGRHITYLEEELADFVLQWMDVGLSSEFLLVLVNLVKFNSCYLDEYIARMVQMICLLCVRTASSVDIEVSLQVLDAVVCYNCLPAESLPLFIVTLCRTINVKELCEPCWKLMRNLLGTHLGHSAIYNMCHLMEDRAYMEDAPLLRGAVFFVGMALWGAHRLYSLRNSPTSVLPSFYQAMACPNEVVSYEIVLSITRLIKKYRKELQVVAWDILLNIIERLLQQLQTLDSPELRTIVHDLLTTVEELCDQNEFHGSQERYFELVERCADQRPESSLLNLISYRAQSIHPAKDGWIQNLQALMESGGGSGGGSGGGSGGGKPILLPNESQSFERSVQLLDQIPSYDTHKIAVLYVGEGQSNSELAILSNEHGSYRYTEFLTGLGRLIELKDCQPDKVYLGGLDVCGEDGQFTYCWHDDIMQAVFHIATLMPTKDVDKHRCDKKRHLGNDFVSIVYNDSGEDFKLGTIKGQFNFVHVIVTPLDYECNLVSLQCRKDMEGLVDTSVAKIVSDRNLPFVARQMALHANMASQVHHSRSNPTDIYPSKWIARLRHIKRLRQRICEEAAYSNPSLPLVHPPSHSKAPAQTPAEPTPGYEVGQRKRLISSVEDFTEFV

SEQ ID NO: 2 - protein, 450 aa, Artificial Sequence
  Synthetic Construct
MAKPTSKDSGLKEKFKILLGLGTPRPNPRSAEGKQTEFIITAEILRELSMECGLNNRIRMIGQICEVAKTKKFEEHAVEALWKAVADLLQPERPLEARHAVLALLKAIVQGQGERLGVLRALFFKVIKDYPSNEDLHERLEVFKALTDNGRHITYLEEELADFVLQWMDVGLSSEFLLVLVNLVKFNSCYLDEYIARMVQMICLLCVRTASSVDIEVSLQVLDAVVCYNCLPAESLPLFIVTLCRTINVKELCEPCWKLMRNLLGTHLGHSAIYNMCHLMEDRAYMEDAPLLRGAVFFVGMALWGAHRLYSLRNSPTSVLPSFYQAMACPNEVVSYEIVLSITRLIKKYRKELQVVAWDILLNIIERLLQQLQTLDSPELRTIVHDLLTTVEELCDQNEFHGSQERYFELVERCADQRPESSLLNLISYRAQSIHPAKDGWIQNLQALME

SEQ ID NO: 3 - protein, 292 aa, Artificial Sequence
  Synthetic Construct
KPILLPNESQSFERSVQLLDQIPSYDTHKIAVLYVGEGQSNSELAILSNEHGSYRYTEFLTGLGRLIELKDCQPDKVYLGGLDVCGEDGQFTYCWHDDIMQAVFHIATLMPTKDVDKHRCDKKRHLGNDFVSIVYNDSGEDFKLGTIKGQFNFVHVIVTPLDYECNLVSLQCRKDMEGLVDTSVAKIVSDRNLPFVARQMALHANMASQVHHSRSNPTDIYPSKWIARLRHIKRLRQRICEEAAYSNPSLPLVHPPSHSKAPAQTPAEPTPGYEVGQRKRLISSVEDFTEFV

SEQ ID NO: 4 - protein, 16 aa, Artificial Sequence
  Synthetic Construct
SGGGSGGGSGGGSGGG

SEQ ID NO: 5 - DNA, 2306 bp, Artificial Sequence
  Synthetic Construct
gctagcactagtaccatggcgaaaccgaccagcaaagatagcggcctgaaagaaaaatttaaaattctgctgggcctgggcaccccgcgcccgaacccgcgcagcgcggaaggcaaacagaccgaatttattattaccgcggaaattctgcgcgaactgagcatggaatgcggcctgaacaaccgcattcgcatgattggccagatttgcgaagtggcgaaaaccaaaaaatttgaagaacatgcggtggaagcgctgtggaaagcggtggcggatctgctgcagccggaacgcccgctggaagcgcgccatgcggtgctggcgctgctgaaagcgattgtgcagggccagggcgaacgcctgggcgtgctgcgcgcgctgttttttaaagtgattaaagattatccgagcaacgaagatctgcatgaacgcctggaagtgtttaaagcgctgaccgataacggccgccatattacctatctggaagaagaactggcggattttgtgctgcagtggatggatgtgggcctgagcagcgaatttctgctggtgctggtgaacctggtgaaatttaacagctgctatctggatgaatatattgcgcgcatggtgcagatgatttgcctgctgtgcgtgcgcaccgcgagcagcgtggatattgaagtgagcctgcaggtgctggatgcggtggtgtgctataactgcctgccggcggaaagcctgccgctgtttattgtgaccctgtgccgcaccattaacgtgaaagaactgtgcgaaccgtgctggaaactgatgcgcaacctgctgggcacccatctgggccatagcgcgatttataacatgtgccatctgatggaagatcgcgcgtatatggaagatgcgccgctgctgcgcggcgcggtgttttttgtgggcatggcgctgtggggcgcgcatcgcctgtatagcctgcgcaacagcccgaccagcgtgctgccgagcttttatcaggcgatggcgtgcccgaacgaagtggtgagctatgaaattgtgctgagcattacccgcctgattaaaaaatatcgcaaagaactgcaggtggtggcgtgggatattctgctgaacattattgaacgcctgctgcagcagctgcagaccctggatagcccggaactgcgcaccattgtgcatgatctgctgaccaccgtggaagaactgtgcgatcagaacgaatttcatggcagccaggaacgctattttgaactggtggaacgctgcgcggatcagcgcccggaaagcagcctgctgaacctgattagctatcgcgcgcagagcattcatccggcgaaagatggctggattcagaacctgcaggcgctgatggaatctggtgggggtagcggaggagggtcagggggcggcagtggaggcggaaaaccgattctgctgccgaacgaaagccagagctttgaacgcagcgtgcagctgctggatcagattccgagctatgatacccataaaattgcggtgctgtatgtgggcgaaggccagagcaacagcgaactggcgattctgagcaacgaacatggcagctatcgctataccgaatttctgaccggcctgggccgcctgattgaactgaaagattgccagccggataaagtgtatctgggcggcctggatgtgtgcggcgaagatggccagtttacctattgctggcatgatgatattatgcaggcggtgtttcatattgcgaccctgatgccgaccaaagatgtggataaacatcgctgcgataaaaaacgccatctgggcaacgattttgtgagcattgtgtataacgatagcggcgaagattttaaactgggcaccattaaaggccagtttaactttgtgcatgtgattgtgaccccgctggattatgaatgcaacctggtgagcctgcagtgccgcaaagatatggaaggcctggtggataccagcgtggcgaaaattgtgagcgatcgcaacctgccgtttgtggcgcgccagatggcgctgcatgcgaacatggcgagccaggtgcatcatagccgcagcaacccgaccgatatttatccgagcaaatggattgcgcgcctgcgccatattaaacgcctgcgccagcgcatttgcgaagaagcggcgtatagcaacccgagcctgccgctggtgcatccgccgagccatagcaaagcgccggcgcagaccccggcggaaccgaccccgggctatgaagtgggccagcgcaaacgcctgattagcagcgtggaagattttaccgaatttgtgtaggcggccgcctcgag

SEQ ID NO: 6 - DNA, 1353 bp, Artificial Sequence
  Synthetic Construct
accatggcgaaaccgaccagcaaagatagcggcctgaaagaaaaatttaaaattctgctgggcctgggcaccccgcgcccgaacccgcgcagcgcggaaggcaaacagaccgaatttattattaccgcggaaattctgcgcgaactgagcatggaatgcggcctgaacaaccgcattcgcatgattggccagatttgcgaagtggcgaaaaccaaaaaatttgaagaacatgcggtggaagcgctgtggaaagcggtggcggatctgctgcagccggaacgcccgctggaagcgcgccatgcggtgctggcgctgctgaaagcgattgtgcagggccagggcgaacgcctgggcgtgctgcgcgcgctgttttttaaagtgattaaagattatccgagcaacgaagatctgcatgaacgcctggaagtgtttaaagcgctgaccgataacggccgccatattacctatctggaagaagaactggcggattttgtgctgcagtggatggatgtgggcctgagcagcgaatttctgctggtgctggtgaacctggtgaaatttaacagctgctatctggatgaatatattgcgcgcatggtgcagatgatttgcctgctgtgcgtgcgcaccgcgagcagcgtggatattgaagtgagcctgcaggtgctggatgcggtggtgtgctataactgcctgccggcggaaagcctgccgctgtttattgtgaccctgtgccgcaccattaacgtgaaagaactgtgcgaaccgtgctggaaactgatgcgcaacctgctgggcacccatctgggccatagcgcgatttataacatgtgccatctgatggaagatcgcgcgtatatggaagatgcgccgctgctgcgcggcgcggtgttttttgtgggcatggcgctgtggggcgcgcatcgcctgtatagcctgcgcaacagcccgaccagcgtgctgccgagcttttatcaggcgatggcgtgcccgaacgaagtggtgagctatgaaattgtgctgagcattacccgcctgattaaaaaatatcgcaaagaactgcaggtggtggcgtgggatattctgctgaacattattgaacgcctgctgcagcagctgcagaccctggatagcccggaactgcgcaccattgtgcatgatctgctgaccaccgtggaagaactgtgcgatcagaacgaatttcatggcagccaggaacgctattttgaactggtggaacgctgcgcggatcagcgcccggaaagcagcctgctgaacctgattagctatcgcgcgcagagcattcatccggcgaaagatggctggattcagaacctgcaggcgctgatggaa

SEQ ID NO: 7 - DNA, 876 bp, Artificial Sequence
  Synthetic Construct
aaaccgattctgctgccgaacgaaagccagagctttgaacgcagcgtgcagctgctggatcagattccgagctatgatacccataaaattgcggtgctgtatgtgggcgaaggccagagcaacagcgaactggcgattctgagcaacgaacatggcagctatcgctataccgaatttctgaccggcctgggccgcctgattgaactgaaagattgccagccggataaagtgtatctgggcggcctggatgtgtgcggcgaagatggccagtttacctattgctggcatgatgatattatgcaggcggtgtttcatattgcgaccctgatgccgaccaaagatgtggataaacatcgctgcgataaaaaacgccatctgggcaacgattttgtgagcattgtgtataacgatagcggcgaagattttaaactgggcaccattaaaggccagtttaactttgtgcatgtgattgtgaccccgctggattatgaatgcaacctggtgagcctgcagtgccgcaaagatatggaaggcctggtggataccagcgtggcgaaaattgtgagcgatcgcaacctgccgtttgtggcgcgccagatggcgctgcatgcgaacatggcgagccaggtgcatcatagccgcagcaacccgaccgatatttatccgagcaaatggattgcgcgcctgcgccatattaaacgcctgcgccagcgcatttgcgaagaagcggcgtatagcaacccgagcctgccgctggtgcatccgccgagccatagcaaagcgccggcgcagaccccggcggaaccgaccccgggctatgaagtgggccagcgcaaacgcctgattagcagcgtggaagattttaccgaatttgtg

SEQ ID NO: 8 - DNA, 48 bp, Artificial Sequence
  Synthetic Construct
tctggtgggggtagcggaggagggtcagggggcggcagtggaggcgga

SEQ ID NO: 9 - DNA, 7540 bp, Artificial Sequence
  Synthetic Construct
ggccgctctagaagataatcaacctctggattacaaaatttgtgaaagattgactggtattcttaactatgttgctccttttacgctatgtggatacgctgctttaatgcctttgtatcatgctattgcttcccgtatggctttcattttctcctccttgtataaatcctggttgctgtctctttatgaggagttgtggcccgttgtcaggcaacgtggcgtggtgtgcactgtgtttgctgacgcaacccccactggttggggcattgccaccacctgtcagctcctttccgggactttcgctttccccctccctattgccacggcggaactcatcgccgcctgccttgcccgctgctggacaggggctcggctgttgggcactgacaattccgtggtgttgtcggggaagctgacgtcctttccatggctgctcgcctgtgttgccacctggattctgcgcgggacgtccttctgctacgtcccttcggccctcaatccagcggaccttccttcccgcggcctgctgccggctctgcggcctcttccgcgtcttcgccttcgccctcagacgagtcggatctccctttgggccgcctccccgcatcggactagagagatccagacatgataagatacattgatgagtttggacaaaccacaactagaatgcagtgaaaaaaatgctttatttgtgaaatttgtgatgctattgctttatttgtaaccattataagctgcaataaacaagttaacaacaacaattgcattcattttatgtttcaggttcagggggaggtgtgggaggttttttagtcgactagagctcgctgatcagcctcgactgtgccttctagttgccagccatctgttgtttgcccctcccccgtgccttccttgaccctggaaggtgccactcccactgtcctttcctaataaaatgaggaaattgcatcgcattgtctgagtaggtgtcattctattctggggggtggggtggggcaggacagcaagggggaggattgggaagacaatagcaggcatgctggggagagatctaggaacccctagtgatggagttggccactccctctctgcgcgctcgctcgctcactgaggccgcccgggcaaagcccgggcgtcgggcgacctttggtcgcccggcctcagtgagcgagcgagcgcgcagagagggagtggccatgcagccagctggcgtaatagcgaagaggcccgcaccgatcgcccttcccaacagttgcgtagcctgaatggcgaatggcgcgacgcgccctgtagcggcgcattaagcgcggcgggtgtggtggttacgcgcagcgtgaccgctacacttgccagcgccctagcgcccgctcctttcgctttcttcccttcctttctcgccacgttcgccggctttccccgtcaagctctaaatcgggggctccctttagggttccgatttagtgctttacggcacctcgaccccaaaaaacttgattagggtgatggttcacgtagtgggccatcgccctgatagacggtttttcgccctttgacgttggagtccacgttctttaatagtggactcttgttccaaactggaacaacactcaaccctatctcggtctattcttttgatttataagggattttgccgatttcggcctattggttaaaaaatgagctgatttaacaaaaatttaacgcgaattttaacaaaatattaacgtttacaatttcctgatgcggtattttctccttacgcatctgtgcggtatttcacaccgcatatggtgcactctcagtacaatctgctctgatgccgcatagttaagccagccccgacacccgccaacacccgctgacgcgccctgacgggcttgtctgctcccggcatccgcttacagacaagctgtgaccgtctccgggagctgcatgtgtcagaggttttcaccgtcatcaccgaaacgcgcgagacgaaagggcctcgtgatacgcctatttttataggttaatgtcatgataataatggtttcttagacgtcaggtggcacttttcggggaaatgtgcgcggaacccctatttgtttatttttctaaatacattcaaatatgtatccgctcatgagacaataaccctgataaatgcttcaataatattgaaaaaggaagagtatgagtattcaacatttccgtgtcgcccttattcccttttttgcggcattttgccttcctgtttttgctcacccagaaacgctggtgaaagtaaaagatgctgaagatcagttgggtgcacgagtgggttacatcgaactggatctcaacagcggtaagatccttgagagttttcgccccgaagaacgttttccaatgatgagcacttttaaagttctgctatgtggcgcggtattatcccgtattgacgccgggcaagagcaactcggtcgccgcatacactattctcagaatgacttggttgagtactcaccagtcacagaaaagcatcttacggatggcatgacagtaagagaattatgcagtgctgccataaccatgagtgataacactgcggccaacttacttctgacaacgatcggaggaccgaaggagctaaccgcttttttgcacaacatgggggatcatgtaactcgccttgatcgttgggaaccggagctgaatgaagccataccaaacgacgagcgtgacaccacgatgcctgtagcaatggcaacaacgttgcgcaaactattaactggcgaactacttactctagcttcccggcaacaattaatagactggatggaggcggataaagttgcaggaccacttctgcgctcggcccttccggctggctggtttattgctgataaatctggagccggtgagcgtgggtctcgcggtatcattgcagcactggggccagatggtaagccctcccgtatcgtagttatctacacgacggggagtcaggcaactatggatgaacgaaatagacagatcgctgagataggtgcctcactgattaagcattggtaactgtcagaccaagtttactcatatatactttagattgatttaaaacttcatttttaatttaaaaggatctaggtgaagatcctttttgataatctcatgaccaaaatcccttaacgtgagttttcgttccactgagcgtcagaccccgtagaaaagatcaaaggatcttcttgagatcctttttttctgcgcgtaatctgctgcttgcaaacaaaaaaaccaccgctaccagcggtggtttgtttgccggatcaagagctaccaactctttttccgaaggtaactggcttcagcagagcgcagataccaaatactgtccttctagtgtagccgtagttaggccaccacttcaagaactctgtagcaccgcctacatacctcgctctgctaatcctgttaccagtggctgctgccagtggcgataagtcgtgtcttaccgggttggactcaagacgatagttaccggataaggcgcagcggtcgggctgaacggggggttcgtgcacacagcccagcttggagcgaacgacctacaccgaactgagatacctacagcgtgagcattgagaaagcgccacgcttcccgaagggagaaaggcggacaggtatccggtaagcggcagggtcggaacaggagagcgcacgagggagcttccagggggaaacgcctggtatctttatagtcctgtcgggtttcgccacctctgacttgagcgtcgatttttgtgatgctcgtcaggggggcggagcctatggaaaaacgccagcaacgcggcctttttacggttcctggccttttgctggccttttgctcacatgttctttcctgcgttatcccctgattctgtggataaccgtattaccgcctttgagtgagctgataccgctcgccgcagccgaacgaccgagcgcagcgagtcagtgagcgaggaagcggaagagcgcccaatacgcaaaccgcctctccccgcgcgttggccgattcattaatgcagctgggctgcaggggggggggggggggggtggggggggggggggggggttggccactccctctctgcgcgctcgctcgctcactgaggccgggcgaccaaaggtcgcccgacgcccgggctttgcccgggcggcctcagtgagcgagcgagcgcgcagagagggagtggccaactccatcactaggggttcctagatctgaattcggtaccctagttattaatagtaatcaattacggggtcattagttcatagcccatatatggagttccgcgttacataacttacggtaaatggcccgcctggctgaccgcccaacgacccccgcccattgacgtcaataatgacgtatgttcccatagtaacgccaatagggactttccattgacgtcaatgggtggactatttacggtaaactgcccacttggcagtacatcaagtgtatcatatgccaagtacgccccctattgacgtcaatgacggtaaatggcccgcctggcattatgcccagtacatgaccttatgggactttcctacttggcagtacatctacgtattagtcatcgctattaccatggtcgaggtgagccccacgttctgcttcactctccccatctcccccccctccccacccccaattttgtatttatttattttttaattattttgtgcagcgatgggggcggggggggggggggggcgcgcgccaggcggggcggggcggggcgaggggcggggcggggcgaggcggagaggtgcggcggcagccaatcagagcggcgcgctccgaaagtttccttttatggcgaggcggcggcggcggcggccctataaaaagcgaagcgcgcggcgggcgggagtcgctgcgacgctgccttcgccccgtgccccgctccgccgccgcctcgcgccgcccgccccggctctgactgaccgcgttactcccacaggtgagcgggcgggacggcccttctcctccgggctgtaattagcgcttggtttaatgacggcttgtttcttttctgtggctgcgtgaaagccttgaggggctccgggagctagagcctctgctaaccatgttcatgccttcttctttttcctacagctcctgggcaacgtgctggttattgtgctgtctcatcattttggcaaagaattcctcgaagatccgaaggggttcaagcttaaaaactagtaccatggcaaaacctacatcaaaagatagcggactgaaagagaagttcaaaatcctgctgggactggggacaccacgccctaatccacggtccgccgagggcaagcagaccgagttcatcatcacagccgagatcctgcgcgagctgtctatggagtgcggcctgaacaatcggatcagaatgatcggccagatttgcgaggtggccaagaccaagaagtttgaggagcacgcagtggaggccctgtggaaggcagtggccgatctgctgcagcctgagagaccactggaggcaaggcacgccgtgctggccctgctgaaggccatcgtgcagggacagggagagcgcctgggcgtgctgcgggccctgttctttaaagtgatcaaggactaccctagcaacgaggatctgcacgagagactggaggtgttcaaggccctgaccgataatggcaggcacatcacatatctggaggaggagctggccgactttgtgctgcagtggatggatgtgggcctgagctccgagttcctgctggtgctggtgaacctggtgaagtttaattcctgctacctggacgagtatatcgcccgcatggtgcagatgatctgcctgctgtgcgtgcggaccgcctctagcgtggacatcgaggtgtctctgcaggtgctggatgccgtggtgtgctacaactgtctgcccgccgagagcctgcctctgttcatcgtgaccctgtgcagaacaatcaatgtgaaggagctgtgcgagccttgttggaagctgatgaggaacctgctgggcacacacctgggacacagcgccatctacaatatgtgccacctgatggaggaccgcgcctatatggaggatgcaccactgctgaggggagccgtgttctttgtgggaatggcactgtggggagcacacagactgtactccctgaggaactctccaaccagcgtgctgccctctttttaccaggctatggcctgtccaaatgaggtggtgtcttatgagatcgtgctgagcatcacacgcctgatcaagaagtatcggaaggagctgcaggtggtggcctgggacatcctgctgaacatcatcgagcgcctgctgcagcagctgcagaccctggacagcccagagctgaggacaatcgtgcacgatctgctgaccacagtggaggagctgtgcgaccagaatgagttccacggctcccaggagcggtactttgagctggtggagcggtgcgcagatcagaggccagagtcctctctgctgaacctgatctcctatcgggcccagtctatccaccctgccaaggacggctggattcagaatctgcaggccctgatggagagcggaggaggctccggaggaggctctggaggcggcagcggcggcggcaagccaatcctgctgcccaacgagagccagagcttcgagcggagcgtgcagctgctggaccagatccccagctacgatacccacaagatcgccgtgctgtatgtgggcgagggccagtctaacagcgagctggccatcctgagcaatgagcacggctcctacagatataccgagtttctgacaggcctgggcaggctgatcgagctgaaggactgccagcccgataaggtgtacctgggaggcctggacgtgtgcggagaggatggccagttcacctattgttggcacgacgatatcatgcaggccgtgtttcacatcgccaccctgatgcctacaaaggacgtggataagcacagatgtgacaagaagaggcacctgggcaacgatttcgtgtccatcgtgtacaatgactctggcgaggacttcaagctgggcaccatcaagggccagttcaactttgtgcacgtgatcgtgacaccactggattatgagtgcaatctggtgagcctgcagtgtagaaaggacatggagggcctggtggataccagcgtggccaagatcgtgtccgacagaaacctgcccttcgtggccaggcagatggccctgcacgccaacatggccagccaggtgcaccactccaggtctaatcctacagacatctacccatccaagtggatcgccaggctgcgccacatcaagcggctgagacagaggatctgcgaggaggccgcctattccaatccctctctgcctctggtgcacccacctagccactccaaggcacctgcacagaccccagcagagccaacaccaggatacgaagtgggacagaggaagcggctgatctcctccgtggaagatttcaccgaatttgtggagcagaagctgattagcgaagaagacctgtaagc

SEQ ID NO: 10 - protein, 1807 aa, Homo sapiens
MAKPTSKDSGLKEKFKILLGLGTPRPNPRSAEGKQTEFIITAEILRELSMECGLNNRIRMIGQICEVAKTKKFEEHAVEALWKAVADLLQPERPLEARHAVLALLKAIVQGQGERLGVLRALFFKVIKDYPSNEDLHERLEVFKALTDNGRHITYLEEELADFVLQWMDVGLSSEFLLVLVNLVKFNSCYLDEYIARMVQMICLLCVRTASSVDIEVSLQVLDAVVCYNCLPAESLPLFIVTLCRTINVKELCEPCWKLMRNLLGTHLGHSAIYNMCHLMEDRAYMEDAPLLRGAVFFVGMALWGAHRLYSLRNSPTSVLPSFYQAMACPNEVVSYEIVLSITRLIKKYRKELQVVAWDILLNIIERLLQQLQTLDSPELRTIVHDLLTTVEELCDQNEFHGSQERYFELVERCADQRPESSLLNLISYRAQSIHPAKDGWIQNLQALMERFFRSESRGAVRIKVLDVLSFVLLINRQFYEEELINSVVISQLSHIPEDKDHQVRKLATQLLVDLAEGCHTHHFNSLLDIIEKVMARSLSPPPELEERDVAAYSASLEDVKTAVLGLLVILQTKLYTLPASHATRVYEMLVSHIQLHYKHSYTLPIASSIRLQAFDFLLLLRADSLHRLGLPNKDGVVRFSPYCVCDYMEPERGSEKKTSGPLSPPTGPPGPAPAGPAVRLGSVPYSLLFRVLLQCLKQESDWKVLKLVLGRLPESLRYKVLIFTSPCSVDQLCSALCSMLSGPKTLERLRGAPEGFSRTDLHLAVVPVLTALISYHNYLDKTKQREMVYCLEQGLIHRCASQCVVALSICSVEMPDIIIKALPVLVVKLTHISATASMAVPLLEFLSTLARLPHLYRNFAAEQYASVFAISLPYTNPSKFNQYIVCLAHHVIAMWFIRCRLPFRKDFVPFITKGLRSNVLLSFDDTPEKDSFRARSTSLNERPKSLRIARPPKQGLNNSPPVKEFKESSAAEAFRCRSISVSEHVVRSRIQTSLTSASLGSADENSVAQADDSLKNLHLELTETCLDMMARYVFSNFTAVPKRSPVGEFLLAGGRTKTWLVGNKLVTVTTSVGTGTRSLLGLDSGELQSGPESSSSPGVHVRQTKEAPAKLESQAGQQVSRGARDRVRSMSGGHGLRVGALDVPASQFLGSATSPGPRTAPAAKPEKASAGTRVPVQEKTNLAAYVPLLTQGWAEILVRRPTGNTSWLMSLENPLSPFSSDINNMPLQELSNALMAAERFKEHRDTALYKSLSVPAASTAKPPPLPRSNTVASFSSLYQSSCQGQLHRSVSWADSAVVMEEGSPGEVPVLVEPPGLEDVEAALGMDRRTDAYSRSSSVSSQEEKSLHAEELVGRGIPIERVVSSEGGRPSVDLSFQPSQPLSKSSSSPELQTLQDILGDPGDKADVGRLSPEVKARSQSGTLDGESAAWSASGEDSRGQPEGPLPSSSPRSPSGLRPRGYTISDSAPSRRGKRVERDALKSRATASNAEKVPGINPSFVFLQLYHSPFFGDESNKPILLPNESQSFERSVQLLDQIPSYDTHKIAVLYVGEGQSNSELAILSNEHGSYRYTEFLTGLGRLIELKDCQPDKVYLGGLDVCGEDGQFTYCWHDDIMQAVFHIATLMPTKDVDKHRCDKKRHLGNDFVSIVYNDSGEDFKLGTIKGQFNFVHVIVTPLDYECNLVSLQCRKDMEGLVDTSVAKIVSDRNLPFVARQMALHANMASQVHHSRSNPTDIYPSKWIARLRHIKRLRQRICEEAAYSNPSLPLVHPPSHSKAPAQTPAEPTPGYEVGQRKRLISSVEDFTEFV

SEQ ID NO: 11 - protein, 768 aa, Artificial Sequence
  Synthetic Construct
MAKPTSKDSGLKEKFKILLGLGTPRPNPRSAEGKQTEFIITAEILRELSMECGLNNRIRMIGQICEVAKTKKFEEHAVEALWKAVADLLQPERPLEARHAVLALLKAIVQGQGERLGVLRALFFKVIKDYPSNEDLHERLEVFKALTDNGRHITYLEEELADFVLQWMDVGLSSEFLLVLVNLVKFNSCYLDEYIARMVQMICLLCVRTASSVDIEVSLQVLDAVVCYNCLPAESLPLFIVTLCRTINVKELCEPCWKLMRNLLGTHLGHSAIYNMCHLMEDRAYMEDAPLLRGAVFFVGMALWGAHRLYSLRNSPTSVLPSFYQAMACPNEVVSYEIVLSITRLIKKYRKELQVVAWDILLNIIERLLQQLQTLDSPELRTIVHDLLTTVEELCDQNEFHGSQERYFELVERCADQRPESSLLNLISYRAQSIHPAKDGWIQNLQALMESGGGSGGGSGGGSGGGKPILLPNESQSFERSVQLLDQIPSYDTHKIAVLYVGEGQSNSELAILSNEHGSYRYTEFLTGLGRLIELKDCQPDKVYLGGLDVCGEDGQFTYCWHDDIMQAVFHIATLMPTKDVDKHRCDKKRHLGNDFVSIVYNDSGEDFKLGTIKGQFNFVHVIVTPLDYECNLVSLQCRKDMEGLVDTSVAKIVSDRNLPFVARQMALHANMASQVHHSRSNPTDIYPSKWIARLRHIKRLRQRICEEAAYSNPSLPLVHPPSHSKAPAQTPAEPTPGYEVGQRKRLISSVEDFTEFVEQKLISEEDL

SEQ ID NO: 12 - DNA, 2336 bp, Artificial Sequence
  Synthetic Construct
gctagcactagtaccatggcgaaaccgaccagcaaagatagcggcctgaaagaaaaatttaaaattctgctgggcctgggcaccccgcgcccgaacccgcgcagcgcggaaggcaaacagaccgaatttattattaccgcggaaattctgcgcgaactgagcatggaatgcggcctgaacaaccgcattcgcatgattggccagatttgcgaagtggcgaaaaccaaaaaatttgaagaacatgcggtggaagcgctgtggaaagcggtggcggatctgctgcagccggaacgcccgctggaagcgcgccatgcggtgctggcgctgctgaaagcgattgtgcagggccagggcgaacgcctgggcgtgctgcgcgcgctgttttttaaagtgattaaagattatccgagcaacgaagatctgcatgaacgcctggaagtgtttaaagcgctgaccgataacggccgccatattacctatctggaagaagaactggcggattttgtgctgcagtggatggatgtgggcctgagcagcgaatttctgctggtgctggtgaacctggtgaaatttaacagctgctatctggatgaatatattgcgcgcatggtgcagatgatttgcctgctgtgcgtgcgcaccgcgagcagcgtggatattgaagtgagcctgcaggtgctggatgcggtggtgtgctataactgcctgccggcggaaagcctgccgctgtttattgtgaccctgtgccgcaccattaacgtgaaagaactgtgcgaaccgtgctggaaactgatgcgcaacctgctgggcacccatctgggccatagcgcgatttataacatgtgccatctgatggaagatcgcgcgtatatggaagatgcgccgctgctgcgcggcgcggtgttttttgtgggcatggcgctgtggggcgcgcatcgcctgtatagcctgcgcaacagcccgaccagcgtgctgccgagcttttatcaggcgatggcgtgcccgaacgaagtggtgagctatgaaattgtgctgagcattacccgcctgattaaaaaatatcgcaaagaactgcaggtggtggcgtgggatattctgctgaacattattgaacgcctgctgcagcagctgcagaccctggatagcccggaactgcgcaccattgtgcatgatctgctgaccaccgtggaagaactgtgcgatcagaacgaatttcatggcagccaggaacgctattttgaactggtggaacgctgcgcggatcagcgcccggaaagcagcctgctgaacctgattagctatcgcgcgcagagcattcatccggcgaaagatggctggattcagaacctgcaggcgctgatggaatctggtgggggtagcggaggagggtcagggggcggcagtggaggcggaaaaccgattctgctgccgaacgaaagccagagctttgaacgcagcgtgcagctgctggatcagattccgagctatgatacccataaaattgcggtgctgtatgtgggcgaaggccagagcaacagcgaactggcgattctgagcaacgaacatggcagctatcgctataccgaatttctgaccggcctgggccgcctgattgaactgaaagattgccagccggataaagtgtatctgggcggcctggatgtgtgcggcgaagatggccagtttacctattgctggcatgatgatattatgcaggcggtgtttcatattgcgaccctgatgccgaccaaagatgtggataaacatcgctgcgataaaaaacgccatctgggcaacgattttgtgagcattgtgtataacgatagcggcgaagattttaaactgggcaccattaaaggccagtttaactttgtgcatgtgattgtgaccccgctggattatgaatgcaacctggtgagcctgcagtgccgcaaagatatggaaggcctggtggataccagcgtggcgaaaattgtgagcgatcgcaacctgccgtttgtggcgcgccagatggcgctgcatgcgaacatggcgagccaggtgcatcatagccgcagcaacccgaccgatatttatccgagcaaatggattgcgcgcctgcgccatattaaacgcctgcgccagcgcatttgcgaagaagcggcgtatagcaacccgagcctgccgctggtgcatccgccgagccatagcaaagcgccggcgcagaccccggcggaaccgaccccgggctatgaagtgggccagcgcaaacgcctgattagcagcgtggaagattttaccgaatttgtggaacaaaaactcatctcagaagaggatctgtaggcggccgcctcgag